European Patent Application EP 4 342 491 A1, published March 27, 2024. Title: HTLV-1 nucleic acid lipid particle vaccine. Applicant: National Institutes of Biomedical Innovation, Health and Nutrition University of the Ryukyus Daiichi Sankyo Company, Limited. The sequence listing filed with the application follows.

SEQUENCE LISTING (40 sequences)

SEQ ID NO: 1 - DNA, 1277 bp, Artificial
  Template plasmid DNA for HTLV-I SU gp46 IVT
gctagcgtaatacgactcactataaggagacccaagctacatttgcttctgacacaactgtgttcactagcaacctcaaacagacaccgccaccatgggcaagttcctggccacactgatcctgttcttccagttctgccccctgatcttcggcgactacagccccagctgctgcaccctgacaatcggcgtgagcagctaccacagcaagccctgcaaccccgcccagcccgtgtgcagctggaccctggacctgctggccctgagcgccgaccaggccctgcagcccccctgccccaacctggtgagctacagcagctaccacgccacctacagcctgtacctgttcccccactggaccaagaagcccaacagaaacggcggaggctactacagcgccagctacagcgacccctgcagcctgaagtgcccctacctgggctgccagagctggacatgcccctacacaggcgccgtgagcagcccctactggaagttccagcacgacgtgaacttcacccaagaggtgagccggctgaacatcaacctgcacttcagcaagtgcggcttcccattcagcctgctggtggacgcccccggctacgaccccatctggttcctgaacaccgagcccagccagctgcccccaacagccccacccctgctgccccacagcaacctggaccacatcctggaacccagcatcccctggaagagcaagctgctgacactggtgcagctgaccctgcagagcaccaactacacctgcatcgtgtgcatcgaccgggccagcctgagcacatggcacgtgctgtacagccccaacgtgagcgtgcccagcagcagcagcacacccctgctgtaccccagcctggcactgcccgccccccacctgacactgcccttcaactggacccactgcttcgacccccagatccaggccatcgtgagcagcccatgccacaacagcctgatcctgcccccattcagcctgagccccgtgcccacactgggcagcagaagcagaagatgagctcgctttcttgctgtccaatttctattaaaggttcctttgttccctaagtccaactactaaactgggggatattatgaagggccttgagcatctggattctgcctaataaaaaacatttattttcattgcaaaaaaaaaaaaaaaaaaaaaaaaaaaaaaaaaaaaaaaaaaaaaaaaaaaaaaaaaaaaaaaaaaaaaaaaaaaaaaaaaaaaaaaaaaaaaaaaaaaaaagagcactagt

SEQ ID NO: 2 - DNA, 24 bp, Artificial
  sense primer
taatacgactcactataaggagac

SEQ ID NO: 3 - DNA, 129 bp, Artificial
  antisense primer
ttttttttttttttttttttttttttttttttttttttttttttttttttttttttttttttttttttttttttttttttttttttttttttttttttttgcaatgaaaataaatgttttttattaggc

SEQ ID NO: 4 - DNA, 1258 bp, Artificial
  Template plasmid DNA for SU gp46 in vitro transcription (IVT)
taatacgactcactataaggagacccaagctacatttgcttctgacacaactgtgttcactagcaacctcaaacagacaccgccaccatgggcaagttcctggccacactgatcctgttcttccagttctgccccctgatcttcggcgactacagccccagctgctgcaccctgacaatcggcgtgagcagctaccacagcaagccctgcaaccccgcccagcccgtgtgcagctggaccctggacctgctggccctgagcgccgaccaggccctgcagcccccctgccccaacctggtgagctacagcagctaccacgccacctacagcctgtacctgttcccccactggaccaagaagcccaacagaaacggcggaggctactacagcgccagctacagcgacccctgcagcctgaagtgcccctacctgggctgccagagctggacatgcccctacacaggcgccgtgagcagcccctactggaagttccagcacgacgtgaacttcacccaagaggtgagccggctgaacatcaacctgcacttcagcaagtgcggcttcccattcagcctgctggtggacgcccccggctacgaccccatctggttcctgaacaccgagcccagccagctgcccccaacagccccacccctgctgccccacagcaacctggaccacatcctggaacccagcatcccctggaagagcaagctgctgacactggtgcagctgaccctgcagagcaccaactacacctgcatcgtgtgcatcgaccgggccagcctgagcacatggcacgtgctgtacagccccaacgtgagcgtgcccagcagcagcagcacacccctgctgtaccccagcctggcactgcccgccccccacctgacactgcccttcaactggacccactgcttcgacccccagatccaggccatcgtgagcagcccatgccacaacagcctgatcctgcccccattcagcctgagccccgtgcccacactgggcagcagaagcagaagatgagctcgctttcttgctgtccaatttctattaaaggttcctttgttccctaagtccaactactaaactgggggatattatgaagggccttgagcatctggattctgcctaataaaaaacatttattttcattgcaaaaaaaaaaaaaaaaaaaaaaaaaaaaaaaaaaaaaaaaaaaaaaaaaaaaaaaaaaaaaaaaaaaaaaaaaaaaaaaaaaaaaaaaaaaaaaaaaaaa

SEQ ID NO: 5 - DNA, 1358 bp, Artificial
  Template plasmid DNA for HTLV-I gp46-Fib IVT
gctagcgtaatacgactcactataaggagacccaagctacatttgcttctgacacaactgtgttcactagcaacctcaaacagacaccgccaccatgggcaagttcctggccacactgatcctgttcttccagttctgccccctgatcttcggcgactacagccccagctgctgcaccctgacaatcggcgtgagcagctaccacagcaagccctgcaaccccgcccagcccgtgtgcagctggaccctggacctgctggccctgagcgccgaccaggccctgcagcccccctgccccaacctggtgagctacagcagctaccacgccacctacagcctgtacctgttcccccactggaccaagaagcccaacagaaacggcggaggctactacagcgccagctacagcgacccctgcagcctgaagtgcccctacctgggctgccagagctggacatgcccctacacaggcgccgtgagcagcccctactggaagttccagcacgacgtgaacttcacccaagaggtgagccggctgaacatcaacctgcacttcagcaagtgcggcttcccattcagcctgctggtggacgcccccggctacgaccccatctggttcctgaacaccgagcccagccagctgcccccaacagccccacccctgctgccccacagcaacctggaccacatcctggaacccagcatcccctggaagagcaagctgctgacactggtgcagctgaccctgcagagcaccaactacacctgcatcgtgtgcatcgaccgggccagcctgagcacatggcacgtgctgtacagccccaacgtgagcgtgcccagcagcagcagcacacccctgctgtaccccagcctggcactgcccgccccccacctgacactgcccttcaactggacccactgcttcgacccccagatccaggccatcgtgagcagcccatgccacaacagcctgatcctgcccccattcagcctgagccccgtgcccacactcggcagcggcagcggcagcggctacatccccgaggcccccagagacggccaggcctacgtcagaaaggacggcgaatgggtgctgctgagcaccttcctgtgagctcgctttcttgctgtccaatttctattaaaggttcctttgttccctaagtccaactactaaactgggggatattatgaagggccttgagcatctggattctgcctaataaaaaacatttattttcattgcaaaaaaaaaaaaaaaaaaaaaaaaaaaaaaaaaaaaaaaaaaaaaaaaaaaaaaaaaaaaaaaaaaaaaaaaaaaaaaaaaaaaaaaaaaaaaaaaaaaaaagagcactagt

SEQ ID NO: 6 - DNA, 1339 bp, Artificial
  Template plasmid DNA for gp46-Fib in vitro transcription (IVT)
taatacgactcactataaggagacccaagctacatttgcttctgacacaactgtgttcactagcaacctcaaacagacaccgccaccatgggcaagttcctggccacactgatcctgttcttccagttctgccccctgatcttcggcgactacagccccagctgctgcaccctgacaatcggcgtgagcagctaccacagcaagccctgcaaccccgcccagcccgtgtgcagctggaccctggacctgctggccctgagcgccgaccaggccctgcagcccccctgccccaacctggtgagctacagcagctaccacgccacctacagcctgtacctgttcccccactggaccaagaagcccaacagaaacggcggaggctactacagcgccagctacagcgacccctgcagcctgaagtgcccctacctgggctgccagagctggacatgcccctacacaggcgccgtgagcagcccctactggaagttccagcacgacgtgaacttcacccaagaggtgagccggctgaacatcaacctgcacttcagcaagtgcggcttcccattcagcctgctggtggacgcccccggctacgaccccatctggttcctgaacaccgagcccagccagctgcccccaacagccccacccctgctgccccacagcaacctggaccacatcctggaacccagcatcccctggaagagcaagctgctgacactggtgcagctgaccctgcagagcaccaactacacctgcatcgtgtgcatcgaccgggccagcctgagcacatggcacgtgctgtacagccccaacgtgagcgtgcccagcagcagcagcacacccctgctgtaccccagcctggcactgcccgccccccacctgacactgcccttcaactggacccactgcttcgacccccagatccaggccatcgtgagcagcccatgccacaacagcctgatcctgcccccattcagcctgagccccgtgcccacactcggcagcggcagcggcagcggctacatccccgaggcccccagagacggccaggcctacgtcagaaaggacggcgaatgggtgctgctgagcaccttcctgtgagctcgctttcttgctgtccaatttctattaaaggttcctttgttccctaagtccaactactaaactgggggatattatgaagggccttgagcatctggattctgcctaataaaaaacatttattttcattgcaaaaaaaaaaaaaaaaaaaaaaaaaaaaaaaaaaaaaaaaaaaaaaaaaaaaaaaaaaaaaaaaaaaaaaaaaaaaaaaaaaaaaaaaaaaaaaaaaaaa

SEQ ID NO: 7 - DNA, 1748 bp, Artificial
  Template plasmid DNA for HTLV-I dgb62-FIb IVT
gctagcgtaatacgactcactataaggagacccaagctacatttgcttctgacacaactgtgttcactagcaacctcaaacagacaccgccaccatgggcaagttcctggccacactgatcctgttcttccagttctgccccctgatcttcggcgactacagccccagctgctgcaccctgacaatcggcgtgagcagctaccacagcaagccctgcaaccccgcccagcccgtgtgcagctggaccctggacctgctggccctgagcgccgaccaggccctgcagcccccctgccccaacctggtgagctacagcagctaccacgccacctacagcctgtacctgttcccccactggaccaagaagcccaacagaaacggcggaggctactacagcgccagctacagcgacccctgcagcctgaagtgcccctacctgggctgccagagctggacatgcccctacacaggcgccgtgagcagcccctactggaagttccagcacgacgtgaacttcacccaagaggtgagccggctgaacatcaacctgcacttcagcaagtgcggcttcccattcagcctgctggtggacgcccccggctacgaccccatctggttcctgaacaccgagcccagccagctgcccccaacagccccacccctgctgccccacagcaacctggaccacatcctggaacccagcatcccctggaagagcaagctgctgacactggtgcagctgaccctgcagagcaccaactacacctgcatcgtgtgcatcgaccgggccagcctgagcacatggcacgtgctgtacagccccaacgtgagcgtgcccagcagcagcagcacacccctgctgtaccccagcctggcactgcccgccccccacctgacactgcccttcaactggacccactgcttcgacccccagatccaggccatcgtgagcagcccatgccacaacagcctgatcctgcccccattcagcctgagccccgtgcccacactcggcagcggaagcggaagcgcagtgcccgtggccgtgtggctggtgagcgccctggccatgggagccggcgtggcaggcggaatcacaggcagcatgagcctggccagcggcaagagcctgctgcacgaggtggacaaggacatcagccagctgacccaggccatcgtgaagaaccacaagaacctgctgaagatcgcccagtacgccgcccagaacagaagaggactggacctgctgttctgggagcaaggcggactgtgcaaagccctccaagagcagtgcagattccccaacatcaccaacagccacgtgcccatcctgcaagagcggcccccactggaaaacagagtgctgacaggatggggcctgaactgggacctgggactgagccagtgggccagagaggccggctacatccccgaggcccccagagacggacaggcctacgtcagaaaggacggcgaatgggtgctgctgagcaccttcctgtgagctcgctttcttgctgtccaatttctattaaaggttcctttgttccctaagtccaactactaaactgggggatattatgaagggccttgagcatctggattctgcctaataaaaaacatttattttcattgcaaaaaaaaaaaaaaaaaaaaaaaaaaaaaaaaaaaaaaaaaaaaaaaaaaaaaaaaaaaaaaaaaaaaaaaaaaaaaaaaaaaaaaaaaaaaaaaaaaaaaagagcactagt

SEQ ID NO: 8 - DNA, 1729 bp, Artificial
  Template plasmid DNA for dgb62-FIb in vitro transcription (IVT)
taatacgactcactataaggagacccaagctacatttgcttctgacacaactgtgttcactagcaacctcaaacagacaccgccaccatgggcaagttcctggccacactgatcctgttcttccagttctgccccctgatcttcggcgactacagccccagctgctgcaccctgacaatcggcgtgagcagctaccacagcaagccctgcaaccccgcccagcccgtgtgcagctggaccctggacctgctggccctgagcgccgaccaggccctgcagcccccctgccccaacctggtgagctacagcagctaccacgccacctacagcctgtacctgttcccccactggaccaagaagcccaacagaaacggcggaggctactacagcgccagctacagcgacccctgcagcctgaagtgcccctacctgggctgccagagctggacatgcccctacacaggcgccgtgagcagcccctactggaagttccagcacgacgtgaacttcacccaagaggtgagccggctgaacatcaacctgcacttcagcaagtgcggcttcccattcagcctgctggtggacgcccccggctacgaccccatctggttcctgaacaccgagcccagccagctgcccccaacagccccacccctgctgccccacagcaacctggaccacatcctggaacccagcatcccctggaagagcaagctgctgacactggtgcagctgaccctgcagagcaccaactacacctgcatcgtgtgcatcgaccgggccagcctgagcacatggcacgtgctgtacagccccaacgtgagcgtgcccagcagcagcagcacacccctgctgtaccccagcctggcactgcccgccccccacctgacactgcccttcaactggacccactgcttcgacccccagatccaggccatcgtgagcagcccatgccacaacagcctgatcctgcccccattcagcctgagccccgtgcccacactcggcagcggaagcggaagcgcagtgcccgtggccgtgtggctggtgagcgccctggccatgggagccggcgtggcaggcggaatcacaggcagcatgagcctggccagcggcaagagcctgctgcacgaggtggacaaggacatcagccagctgacccaggccatcgtgaagaaccacaagaacctgctgaagatcgcccagtacgccgcccagaacagaagaggactggacctgctgttctgggagcaaggcggactgtgcaaagccctccaagagcagtgcagattccccaacatcaccaacagccacgtgcccatcctgcaagagcggcccccactggaaaacagagtgctgacaggatggggcctgaactgggacctgggactgagccagtgggccagagaggccggctacatccccgaggcccccagagacggacaggcctacgtcagaaaggacggcgaatgggtgctgctgagcaccttcctgtgagctcgctttcttgctgtccaatttctattaaaggttcctttgttccctaagtccaactactaaactgggggatattatgaagggccttgagcatctggattctgcctaataaaaaacatttattttcattgcaaaaaaaaaaaaaaaaaaaaaaaaaaaaaaaaaaaaaaaaaaaaaaaaaaaaaaaaaaaaaaaaaaaaaaaaaaaaaaaaaaaaaaaaaaaaaaaaaaaa

SEQ ID NO: 9 - DNA, 1451 bp, Artificial
  Template plasmid DNA for HTLV-I sec Tax mutant IVT
gctagcgtaatacgactcactataaggagacccaagctacatttgcttctgacacaactgtgttcactagcaacctcaaacagacaccgccaccatggactggacctggatcctgttcctggtggccgccgccacaagagtgcacagcgcacacttcccaggcttcggccagagcctgctgttcggctaccccgtgtacgtgttcggcgactgcgtgcaaggcgactggtgccccatcagcggcggcctgtgcagcgccagactgcacagacacgccctgctggccacatgccccgagcaccagatcacctgggaccccatcgacggcagagtgatcggaagcgccctgcagttcctgatccccagactgcccagcttccccacacagagaaccagcaagaccctgaaggtgctgaccccccccatcacacacaccacacccaacatccccccaagcttcctgcaggccatgcggaagtacagccccttcagaaacggctacatggaacccacactgggccagcacctgcccgccagcagcttccccgaccccggactgaggccccagaacctgtacacactgtggggcggcagcgtcgtgtgcatgtacctgtaccagctgagcccaccaatcacatggcccctgctgccccacgtgatcttctgccaccccggacagctgggcgccttcctgaccaacgtgccctacaagcggatcgaggaactgctgtacaagatcagcctgaccacaggcgccctgatcatcctgcccgaggactgcctgcccaccacactgttccagcccgccagagcccccgtgacactgaccgcctggcagaacggcctgctgccattccacagcaccctgacaacacccggcctgatctggaccttcaccgacggcacacccatgatcagcggcccctgccccaaggacggccagcccagcctggtgctgcagagcagcagcttcatcttccacaagttccagaccaaggcctaccaccccagcttcctgctgagccacggactgatccagtacagcagcttccacagcctgcacctgctgttcgaagagtacacaaacatccccatcagccggagcttcaacgagaaagaggccgacgacaacgaccacgagccccagatcagccccggcggactggaaccccccagcgagaagcacttccgggaaaccgaagtgtgagctcgctttcttgctgtccaatttctattaaaggttcctttgttccctaagtccaactactaaactgggggatattatgaagggccttgagcatctggattctgcctaataaaaaacatttattttcattgcaaaaaaaaaaaaaaaaaaaaaaaaaaaaaaaaaaaaaaaaaaaaaaaaaaaaaaaaaaaaaaaaaaaaaaaaaaaaaaaaaaaaaaaaaaaaaaaaaaaaaagagcactagt

SEQ ID NO: 10 - DNA, 1432 bp, Artificial
  Template plasmid DNA for sec Tax mutant in vitro transcription (IVT)
taatacgactcactataaggagacccaagctacatttgcttctgacacaactgtgttcactagcaacctcaaacagacaccgccaccatggactggacctggatcctgttcctggtggccgccgccacaagagtgcacagcgcacacttcccaggcttcggccagagcctgctgttcggctaccccgtgtacgtgttcggcgactgcgtgcaaggcgactggtgccccatcagcggcggcctgtgcagcgccagactgcacagacacgccctgctggccacatgccccgagcaccagatcacctgggaccccatcgacggcagagtgatcggaagcgccctgcagttcctgatccccagactgcccagcttccccacacagagaaccagcaagaccctgaaggtgctgaccccccccatcacacacaccacacccaacatccccccaagcttcctgcaggccatgcggaagtacagccccttcagaaacggctacatggaacccacactgggccagcacctgcccgccagcagcttccccgaccccggactgaggccccagaacctgtacacactgtggggcggcagcgtcgtgtgcatgtacctgtaccagctgagcccaccaatcacatggcccctgctgccccacgtgatcttctgccaccccggacagctgggcgccttcctgaccaacgtgccctacaagcggatcgaggaactgctgtacaagatcagcctgaccacaggcgccctgatcatcctgcccgaggactgcctgcccaccacactgttccagcccgccagagcccccgtgacactgaccgcctggcagaacggcctgctgccattccacagcaccctgacaacacccggcctgatctggaccttcaccgacggcacacccatgatcagcggcccctgccccaaggacggccagcccagcctggtgctgcagagcagcagcttcatcttccacaagttccagaccaaggcctaccaccccagcttcctgctgagccacggactgatccagtacagcagcttccacagcctgcacctgctgttcgaagagtacacaaacatccccatcagccggagcttcaacgagaaagaggccgacgacaacgaccacgagccccagatcagccccggcggactggaaccccccagcgagaagcacttccgggaaaccgaagtgtgagctcgctttcttgctgtccaatttctattaaaggttcctttgttccctaagtccaactactaaactgggggatattatgaagggccttgagcatctggattctgcctaataaaaaacatttattttcattgcaaaaaaaaaaaaaaaaaaaaaaaaaaaaaaaaaaaaaaaaaaaaaaaaaaaaaaaaaaaaaaaaaaaaaaaaaaaaaaaaaaaaaaaaaaaaaaaaaaaa

SEQ ID NO: 11 - protein, 353 aa, Artificial
  Tax wild-type amino acid sequence
MAHFPGFGQSLLFGYPVYVFGDCVQGDWCPISGGLCSARLHRHALLATCPEHQITWDPIDGRVIGSALQFLIPRLPSFPTQRTSKTLKVLTPPITHTTPNIPPSFLQAMRKYSPFRNGYMEPTLGQHLPTLSFPDPGLRPQNLYTLWGGSVVCMYLYQLSPPITWPLLPHVIFCHPGQLGAFLTNVPYKRIEELLYKISLTTGALIILPEDCLPTTLFQPARAPVTLTAWQNGLLPFHSTLTTPGLIWTFTDGTPMISGPCPKDGQPSLVLQSSSFIFHKFQTKAYHPSFLLSHGLIQYSSFHSLHLLFEEYTNIPISLLFNEKEADDNDHEPQISPGGLEPPSEKHFRETEV

SEQ ID NO: 12 - protein, 353 aa, Artificial
  Tax mutant (T130A/L131S/L319R/L320S) amino acid sequence
MAHFPGFGQSLLFGYPVYVFGDCVQGDWCPISGGLCSARLHRHALLATCPEHQITWDPIDGRVIGSALQFLIPRLPSFPTQRTSKTLKVLTPPITHTTPNIPPSFLQAMRKYSPFRNGYMEPTLGQHLPASSFPDPGLRPQNLYTLWGGSVVCMYLYQLSPPITWPLLPHVIFCHPGQLGAFLTNVPYKRIEELLYKISLTTGALIILPEDCLPTTLFQPARAPVTLTAWQNGLLPFHSTLTTPGLIWTFTDGTPMISGPCPKDGQPSLVLQSSSFIFHKFQTKAYHPSFLLSHGLIQYSSFHSLHLLFEEYTNIPISRSFNEKEADDNDHEPQISPGGLEPPSEKHFRETEV

SEQ ID NO: 13 - protein, 370 aa, Artificial
  Secretory Tax mutant (T130A/L131S/L319R/L320S) amino acid sequence
MDWTWILFLVAAATRVHSAHFPGFGQSLLFGYPVYVFGDCVQGDWCPISGGLCSARLHRHALLATCPEHQITWDPIDGRVIGSALQFLIPRLPSFPTQRTSKTLKVLTPPITHTTPNIPPSFLQAMRKYSPFRNGYMEPTLGQHLPASSFPDPGLRPQNLYTLWGGSVVCMYLYQLSPPITWPLLPHVIFCHPGQLGAFLTNVPYKRIEELLYKISLTTGALIILPEDCLPTTLFQPARAPVTLTAWQNGLLPFHSTLTTPGLIWTFTDGTPMISGPCPKDGQPSLVLQSSSFIFHKFQTKAYHPSFLLSHGLIQYSSFHSLHLLFEEYTNIPISRSFNEKEADDNDHEPQISPGGLEPPSEKHFRETEV

SEQ ID NO: 14 - protein, 312 aa, Artificial
  gp46 amino acid sequence
MGKFLATLILFFQFCPLIFGDYSPSCCTLTIGVSSYHSKPCNPAQPVCSWTLDLLALSADQALQPPCPNLVSYSSYHATYSLYLFPHWTKKPNRNGGGYYSASYSDPCSLKCPYLGCQSWTCPYTGAVSSPYWKFQHDVNFTQEVSRLNINLHFSKCGFPFSLLVDAPGYDPIWFLNTEPSQLPPTAPPLLPHSNLDHILEPSIPWKSKLLTLVQLTLQSTNYTCIVCIDRASLSTWHVLYSPNVSVPSSSSTPLLYPSLALPAPHLTLPFNWTHCFDPQIQAIVSSPCHNSLILPPFSLSPVPTLGSRSRR

SEQ ID NO: 15 - protein, 339 aa, Artificial
  gp46-Fib amino acid sequence
MGKFLATLILFFQFCPLIFGDYSPSCCTLTIGVSSYHSKPCNPAQPVCSWTLDLLALSADQALQPPCPNLVSYSSYHATYSLYLFPHWTKKPNRNGGGYYSASYSDPCSLKCPYLGCQSWTCPYTGAVSSPYWKFQHDVNFTQEVSRLNINLHFSKCGFPFSLLVDAPGYDPIWFLNTEPSQLPPTAPPLLPHSNLDHILEPSIPWKSKLLTLVQLTLQSTNYTCIVCIDRASLSTWHVLYSPNVSVPSSSSTPLLYPSLALPAPHLTLPFNWTHCFDPQIQAIVSSPCHNSLILPPFSLSPVPTLGSGSGSGYIPEAPRDGQAYVRKDGEWVLLSTFL

SEQ ID NO: 16 - protein, 469 aa, Artificial
  dgp62 amino acid sequence
MGKFLATLILFFQFCPLIFGDYSPSCCTLTIGVSSYHSKPCNPAQPVCSWTLDLLALSADQALQPPCPNLVSYSSYHATYSLYLFPHWTKKPNRNGGGYYSASYSDPCSLKCPYLGCQSWTCPYTGAVSSPYWKFQHDVNFTQEVSRLNINLHFSKCGFPFSLLVDAPGYDPIWFLNTEPSQLPPTAPPLLPHSNLDHILEPSIPWKSKLLTLVQLTLQSTNYTCIVCIDRASLSTWHVLYSPNVSVPSSSSTPLLYPSLALPAPHLTLPFNWTHCFDPQIQAIVSSPCHNSLILPPFSLSPVPTLGSGSGSAVPVAVWLVSALAMGAGVAGGITGSMSLASGKSLLHEVDKDISQLTQAIVKNHKNLLKIAQYAAQNRRGLDLLFWEQGGLCKALQEQCRFPNITNSHVPILQERPPLENRVLTGWGLNWDLGLSQWAREAGYIPEAPRDGQAYVRKDGEWVLLSTFL

SEQ ID NO: 17 - RNA, 1241 nt, Artificial
  SU gp46 mRNA
aggagacccaagcuacauuugcuucugacacaacuguguucacuagcaaccucaaacagacaccgccaccaugggcaaguuccuggccacacugauccuguucuuccaguucugcccccugaucuucggcgacuacagccccagcugcugcacccugacaaucggcgugagcagcuaccacagcaagcccugcaaccccgcccagcccgugugcagcuggacccuggaccugcuggcccugagcgccgaccaggcccugcagccccccugccccaaccuggugagcuacagcagcuaccacgccaccuacagccuguaccuguucccccacuggaccaagaagcccaacagaaacggcggaggcuacuacagcgccagcuacagcgaccccugcagccugaagugccccuaccugggcugccagagcuggacaugccccuacacaggcgccgugagcagccccuacuggaaguuccagcacgacgugaacuucacccaagaggugagccggcugaacaucaaccugcacuucagcaagugcggcuucccauucagccugcugguggacgcccccggcuacgaccccaucugguuccugaacaccgagcccagccagcugcccccaacagccccaccccugcugccccacagcaaccuggaccacauccuggaacccagcauccccuggaagagcaagcugcugacacuggugcagcugacccugcagagcaccaacuacaccugcaucgugugcaucgaccgggccagccugagcacauggcacgugcuguacagccccaacgugagcgugcccagcagcagcagcacaccccugcuguaccccagccuggcacugcccgccccccaccugacacugcccuucaacuggacccacugcuucgacccccagauccaggccaucgugagcagcccaugccacaacagccugauccugcccccauucagccugagccccgugcccacacugggcagcagaagcagaagaugagcucgcuuucuugcuguccaauuucuauuaaagguuccuuuguucccuaaguccaacuacuaaacugggggauauuaugaagggccuugagcaucuggauucugccuaauaaaaaacauuuauuuucauugcaaaaaaaaaaaaaaaaaaaaaaaaaaaaaaaaaaaaaaaaaaaaaaaaaaaaaaaaaaaaaaaaaaaaaaaaaaaaaaaaaaaaaaaaaaaaaaaaaaaa

SEQ ID NO: 18 - RNA, 1322 nt, Artificial
  gp46-Fib mRNA
aggagacccaagcuacauuugcuucugacacaacuguguucacuagcaaccucaaacagacaccgccaccaugggcaaguuccuggccacacugauccuguucuuccaguucugcccccugaucuucggcgacuacagccccagcugcugcacccugacaaucggcgugagcagcuaccacagcaagcccugcaaccccgcccagcccgugugcagcuggacccuggaccugcuggcccugagcgccgaccaggcccugcagccccccugccccaaccuggugagcuacagcagcuaccacgccaccuacagccuguaccuguucccccacuggaccaagaagcccaacagaaacggcggaggcuacuacagcgccagcuacagcgaccccugcagccugaagugccccuaccugggcugccagagcuggacaugccccuacacaggcgccgugagcagccccuacuggaaguuccagcacgacgugaacuucacccaagaggugagccggcugaacaucaaccugcacuucagcaagugcggcuucccauucagccugcugguggacgcccccggcuacgaccccaucugguuccugaacaccgagcccagccagcugcccccaacagccccaccccugcugccccacagcaaccuggaccacauccuggaacccagcauccccuggaagagcaagcugcugacacuggugcagcugacccugcagagcaccaacuacaccugcaucgugugcaucgaccgggccagccugagcacauggcacgugcuguacagccccaacgugagcgugcccagcagcagcagcacaccccugcuguaccccagccuggcacugcccgccccccaccugacacugcccuucaacuggacccacugcuucgacccccagauccaggccaucgugagcagcccaugccacaacagccugauccugcccccauucagccugagccccgugcccacacucggcagcggcagcggcagcggcuacauccccgaggcccccagagacggccaggccuacgucagaaaggacggcgaaugggugcugcugagcaccuuccugugagcucgcuuucuugcuguccaauuucuauuaaagguuccuuuguucccuaaguccaacuacuaaacugggggauauuaugaagggccuugagcaucuggauucugccuaauaaaaaacauuuauuuucauugcaaaaaaaaaaaaaaaaaaaaaaaaaaaaaaaaaaaaaaaaaaaaaaaaaaaaaaaaaaaaaaaaaaaaaaaaaaaaaaaaaaaaaaaaaaaaaaaaaaaa

SEQ ID NO: 19 - RNA, 1712 nt, Artificial
  dgp62-Fib mRNA
aggagacccaagcuacauuugcuucugacacaacuguguucacuagcaaccucaaacagacaccgccaccaugggcaaguuccuggccacacugauccuguucuuccaguucugcccccugaucuucggcgacuacagccccagcugcugcacccugacaaucggcgugagcagcuaccacagcaagcccugcaaccccgcccagcccgugugcagcuggacccuggaccugcuggcccugagcgccgaccaggcccugcagccccccugccccaaccuggugagcuacagcagcuaccacgccaccuacagccuguaccuguucccccacuggaccaagaagcccaacagaaacggcggaggcuacuacagcgccagcuacagcgaccccugcagccugaagugccccuaccugggcugccagagcuggacaugccccuacacaggcgccgugagcagccccuacuggaaguuccagcacgacgugaacuucacccaagaggugagccggcugaacaucaaccugcacuucagcaagugcggcuucccauucagccugcugguggacgcccccggcuacgaccccaucugguuccugaacaccgagcccagccagcugcccccaacagccccaccccugcugccccacagcaaccuggaccacauccuggaacccagcauccccuggaagagcaagcugcugacacuggugcagcugacccugcagagcaccaacuacaccugcaucgugugcaucgaccgggccagccugagcacauggcacgugcuguacagccccaacgugagcgugcccagcagcagcagcacaccccugcuguaccccagccuggcacugcccgccccccaccugacacugcccuucaacuggacccacugcuucgacccccagauccaggccaucgugagcagcccaugccacaacagccugauccugcccccauucagccugagccccgugcccacacucggcagcggaagcggaagcgcagugcccguggccguguggcuggugagcgcccuggccaugggagccggcguggcaggcggaaucacaggcagcaugagccuggccagcggcaagagccugcugcacgagguggacaaggacaucagccagcugacccaggccaucgugaagaaccacaagaaccugcugaagaucgcccaguacgccgcccagaacagaagaggacuggaccugcuguucugggagcaaggcggacugugcaaagcccuccaagagcagugcagauuccccaacaucaccaacagccacgugcccauccugcaagagcggcccccacuggaaaacagagugcugacaggauggggccugaacugggaccugggacugagccagugggccagagaggccggcuacauccccgaggcccccagagacggacaggccuacgucagaaaggacggcgaaugggugcugcugagcaccuuccugugagcucgcuuucuugcuguccaauuucuauuaaagguuccuuuguucccuaaguccaacuacuaaacugggggauauuaugaagggccuugagcaucuggauucugccuaauaaaaaacauuuauuuucauugcaaaaaaaaaaaaaaaaaaaaaaaaaaaaaaaaaaaaaaaaaaaaaaaaaaaaaaaaaaaaaaaaaaaaaaaaaaaaaaaaaaaaaaaaaaaaaaaaaaaa

SEQ ID NO: 20 - RNA, 1415 nt, Artificial
  sec Tax mutant mRNA
aggagacccaagcuacauuugcuucugacacaacuguguucacuagcaaccucaaacagacaccgccaccauggacuggaccuggauccuguuccugguggccgccgccacaagagugcacagcgcacacuucccaggcuucggccagagccugcuguucggcuaccccguguacguguucggcgacugcgugcaaggcgacuggugccccaucagcggcggccugugcagcgccagacugcacagacacgcccugcuggccacaugccccgagcaccagaucaccugggaccccaucgacggcagagugaucggaagcgcccugcaguuccugauccccagacugcccagcuuccccacacagagaaccagcaagacccugaaggugcugaccccccccaucacacacaccacacccaacauccccccaagcuuccugcaggccaugcggaaguacagccccuucagaaacggcuacauggaacccacacugggccagcaccugcccgccagcagcuuccccgaccccggacugaggccccagaaccuguacacacuguggggcggcagcgucgugugcauguaccuguaccagcugagcccaccaaucacauggccccugcugccccacgugaucuucugccaccccggacagcugggcgccuuccugaccaacgugcccuacaagcggaucgaggaacugcuguacaagaucagccugaccacaggcgcccugaucauccugcccgaggacugccugcccaccacacuguuccagcccgccagagcccccgugacacugaccgccuggcagaacggccugcugccauuccacagcacccugacaacacccggccugaucuggaccuucaccgacggcacacccaugaucagcggccccugccccaaggacggccagcccagccuggugcugcagagcagcagcuucaucuuccacaaguuccagaccaaggccuaccaccccagcuuccugcugagccacggacugauccaguacagcagcuuccacagccugcaccugcuguucgaagaguacacaaacauccccaucagccggagcuucaacgagaaagaggccgacgacaacgaccacgagccccagaucagccccggcggacuggaaccccccagcgagaagcacuuccgggaaaccgaagugugagcucgcuuucuugcuguccaauuucuauuaaagguuccuuuguucccuaaguccaacuacuaaacugggggauauuaugaagggccuugagcaucuggauucugccuaauaaaaaacauuuauuuucauugcaaaaaaaaaaaaaaaaaaaaaaaaaaaaaaaaaaaaaaaaaaaaaaaaaaaaaaaaaaaaaaaaaaaaaaaaaaaaaaaaaaaaaaaaaaaaaaaaaaaa

SEQ ID NO: 21 - DNA, 1349 bp, Artificial
  Template DNA nucleotide sequence for gp46-Fib  polyA95
gctagcgtaatacgactcactataaggagacccaagctacatttgcttctgacacaactgtgttcactagcaacctcaaacagacaccgccaccatgggcaagttcctggccacactgatcctgttcttccagttctgccccctgatcttcggcgactacagccccagctgctgcaccctgacaatcggcgtgagcagctaccacagcaagccctgcaaccccgcccagcccgtgtgcagctggaccctggacctgctggccctgagcgccgaccaggccctgcagcccccctgccccaacctggtgagctacagcagctaccacgccacctacagcctgtacctgttcccccactggaccaagaagcccaacagaaacggcggaggctactacagcgccagctacagcgacccctgcagcctgaagtgcccctacctgggctgccagagctggacatgcccctacacaggcgccgtgagcagcccctactggaagttccagcacgacgtgaacttcacccaagaggtgagccggctgaacatcaacctgcacttcagcaagtgcggcttcccattcagcctgctggtggacgcccccggctacgaccccatctggttcctgaacaccgagcccagccagctgcccccaacagccccacccctgctgccccacagcaacctggaccacatcctggaacccagcatcccctggaagagcaagctgctgacactggtgcagctgaccctgcagagcaccaactacacctgcatcgtgtgcatcgaccgggccagcctgagcacatggcacgtgctgtacagccccaacgtgagcgtgcccagcagcagcagcacacccctgctgtaccccagcctggcactgcccgccccccacctgacactgcccttcaactggacccactgcttcgacccccagatccaggccatcgtgagcagcccatgccacaacagcctgatcctgcccccattcagcctgagccccgtgcccacactcggcagcggcagcggcagcggctacatccccgaggcccccagagacggccaggcctacgtcagaaaggacggcgaatgggtgctgctgagcaccttcctgtgagctcgctttcttgctgtccaatttctattaaaggttcctttgttccctaagtccaactactaaactgggggatattatgaagggccttgagcatctggattctgcctaataaaaaacatttattttcattgcaaaaaaaaaaaaaaaaaaaaaaaaaaaaaaaaaaaaaaaaaaaaaaaaaaaaaaaaaaaaaaaaaaaaaaaaaaaaaaaaaaaaaaaaaaaaaaacgaagagc

SEQ ID NO: 22 - DNA, 1334 bp, Artificial
  Template DNA nucleotide sequence for gp46-Fib  polyA80
gctagcgtaatacgactcactataaggagacccaagctacatttgcttctgacacaactgtgttcactagcaacctcaaacagacaccgccaccatgggcaagttcctggccacactgatcctgttcttccagttctgccccctgatcttcggcgactacagccccagctgctgcaccctgacaatcggcgtgagcagctaccacagcaagccctgcaaccccgcccagcccgtgtgcagctggaccctggacctgctggccctgagcgccgaccaggccctgcagcccccctgccccaacctggtgagctacagcagctaccacgccacctacagcctgtacctgttcccccactggaccaagaagcccaacagaaacggcggaggctactacagcgccagctacagcgacccctgcagcctgaagtgcccctacctgggctgccagagctggacatgcccctacacaggcgccgtgagcagcccctactggaagttccagcacgacgtgaacttcacccaagaggtgagccggctgaacatcaacctgcacttcagcaagtgcggcttcccattcagcctgctggtggacgcccccggctacgaccccatctggttcctgaacaccgagcccagccagctgcccccaacagccccacccctgctgccccacagcaacctggaccacatcctggaacccagcatcccctggaagagcaagctgctgacactggtgcagctgaccctgcagagcaccaactacacctgcatcgtgtgcatcgaccgggccagcctgagcacatggcacgtgctgtacagccccaacgtgagcgtgcccagcagcagcagcacacccctgctgtaccccagcctggcactgcccgccccccacctgacactgcccttcaactggacccactgcttcgacccccagatccaggccatcgtgagcagcccatgccacaacagcctgatcctgcccccattcagcctgagccccgtgcccacactcggcagcggcagcggcagcggctacatccccgaggcccccagagacggccaggcctacgtcagaaaggacggcgaatgggtgctgctgagcaccttcctgtgagctcgctttcttgctgtccaatttctattaaaggttcctttgttccctaagtccaactactaaactgggggatattatgaagggccttgagcatctggattctgcctaataaaaaacatttattttcattgcaaaaaaaaaaaaaaaaaaaaaaaaaaaaaaaaaaaaaaaaaaaaaaaaaaaaaaaaaaaaaaaaaaaaaaaaaaaaaaaacgaagagc

SEQ ID NO: 23 - DNA, 1314 bp, Artificial
  Template DNA nucleotide sequence for gp46-Fib  polyA60
gctagcgtaatacgactcactataaggagacccaagctacatttgcttctgacacaactgtgttcactagcaacctcaaacagacaccgccaccatgggcaagttcctggccacactgatcctgttcttccagttctgccccctgatcttcggcgactacagccccagctgctgcaccctgacaatcggcgtgagcagctaccacagcaagccctgcaaccccgcccagcccgtgtgcagctggaccctggacctgctggccctgagcgccgaccaggccctgcagcccccctgccccaacctggtgagctacagcagctaccacgccacctacagcctgtacctgttcccccactggaccaagaagcccaacagaaacggcggaggctactacagcgccagctacagcgacccctgcagcctgaagtgcccctacctgggctgccagagctggacatgcccctacacaggcgccgtgagcagcccctactggaagttccagcacgacgtgaacttcacccaagaggtgagccggctgaacatcaacctgcacttcagcaagtgcggcttcccattcagcctgctggtggacgcccccggctacgaccccatctggttcctgaacaccgagcccagccagctgcccccaacagccccacccctgctgccccacagcaacctggaccacatcctggaacccagcatcccctggaagagcaagctgctgacactggtgcagctgaccctgcagagcaccaactacacctgcatcgtgtgcatcgaccgggccagcctgagcacatggcacgtgctgtacagccccaacgtgagcgtgcccagcagcagcagcacacccctgctgtaccccagcctggcactgcccgccccccacctgacactgcccttcaactggacccactgcttcgacccccagatccaggccatcgtgagcagcccatgccacaacagcctgatcctgcccccattcagcctgagccccgtgcccacactcggcagcggcagcggcagcggctacatccccgaggcccccagagacggccaggcctacgtcagaaaggacggcgaatgggtgctgctgagcaccttcctgtgagctcgctttcttgctgtccaatttctattaaaggttcctttgttccctaagtccaactactaaactgggggatattatgaagggccttgagcatctggattctgcctaataaaaaacatttattttcattgcaaaaaaaaaaaaaaaaaaaaaaaaaaaaaaaaaaaaaaaaaaaaaaaaaaaaaaaaaaaacgaagagc

SEQ ID NO: 24 - DNA, 1294 bp, Artificial
  Template DNA nucleotide sequence for gp46-Fib  polyA40
gctagcgtaatacgactcactataaggagacccaagctacatttgcttctgacacaactgtgttcactagcaacctcaaacagacaccgccaccatgggcaagttcctggccacactgatcctgttcttccagttctgccccctgatcttcggcgactacagccccagctgctgcaccctgacaatcggcgtgagcagctaccacagcaagccctgcaaccccgcccagcccgtgtgcagctggaccctggacctgctggccctgagcgccgaccaggccctgcagcccccctgccccaacctggtgagctacagcagctaccacgccacctacagcctgtacctgttcccccactggaccaagaagcccaacagaaacggcggaggctactacagcgccagctacagcgacccctgcagcctgaagtgcccctacctgggctgccagagctggacatgcccctacacaggcgccgtgagcagcccctactggaagttccagcacgacgtgaacttcacccaagaggtgagccggctgaacatcaacctgcacttcagcaagtgcggcttcccattcagcctgctggtggacgcccccggctacgaccccatctggttcctgaacaccgagcccagccagctgcccccaacagccccacccctgctgccccacagcaacctggaccacatcctggaacccagcatcccctggaagagcaagctgctgacactggtgcagctgaccctgcagagcaccaactacacctgcatcgtgtgcatcgaccgggccagcctgagcacatggcacgtgctgtacagccccaacgtgagcgtgcccagcagcagcagcacacccctgctgtaccccagcctggcactgcccgccccccacctgacactgcccttcaactggacccactgcttcgacccccagatccaggccatcgtgagcagcccatgccacaacagcctgatcctgcccccattcagcctgagccccgtgcccacactcggcagcggcagcggcagcggctacatccccgaggcccccagagacggccaggcctacgtcagaaaggacggcgaatgggtgctgctgagcaccttcctgtgagctcgctttcttgctgtccaatttctattaaaggttcctttgttccctaagtccaactactaaactgggggatattatgaagggccttgagcatctggattctgcctaataaaaaacatttattttcattgcaaaaaaaaaaaaaaaaaaaaaaaaaaaaaaaaaaaaaaaacgaagagc

SEQ ID NO: 25 - DNA, 1274 bp, Artificial
  Template DNA nucleotide sequence for gp46-Fib  polyA20
gctagcgtaatacgactcactataaggagacccaagctacatttgcttctgacacaactgtgttcactagcaacctcaaacagacaccgccaccatgggcaagttcctggccacactgatcctgttcttccagttctgccccctgatcttcggcgactacagccccagctgctgcaccctgacaatcggcgtgagcagctaccacagcaagccctgcaaccccgcccagcccgtgtgcagctggaccctggacctgctggccctgagcgccgaccaggccctgcagcccccctgccccaacctggtgagctacagcagctaccacgccacctacagcctgtacctgttcccccactggaccaagaagcccaacagaaacggcggaggctactacagcgccagctacagcgacccctgcagcctgaagtgcccctacctgggctgccagagctggacatgcccctacacaggcgccgtgagcagcccctactggaagttccagcacgacgtgaacttcacccaagaggtgagccggctgaacatcaacctgcacttcagcaagtgcggcttcccattcagcctgctggtggacgcccccggctacgaccccatctggttcctgaacaccgagcccagccagctgcccccaacagccccacccctgctgccccacagcaacctggaccacatcctggaacccagcatcccctggaagagcaagctgctgacactggtgcagctgaccctgcagagcaccaactacacctgcatcgtgtgcatcgaccgggccagcctgagcacatggcacgtgctgtacagccccaacgtgagcgtgcccagcagcagcagcacacccctgctgtaccccagcctggcactgcccgccccccacctgacactgcccttcaactggacccactgcttcgacccccagatccaggccatcgtgagcagcccatgccacaacagcctgatcctgcccccattcagcctgagccccgtgcccacactcggcagcggcagcggcagcggctacatccccgaggcccccagagacggccaggcctacgtcagaaaggacggcgaatgggtgctgctgagcaccttcctgtgagctcgctttcttgctgtccaatttctattaaaggttcctttgttccctaagtccaactactaaactgggggatattatgaagggccttgagcatctggattctgcctaataaaaaacatttattttcattgcaaaaaaaaaaaaaaaaaaaacgaagagc

SEQ ID NO: 26 - DNA, 1442 bp, Artificial
  Template DNA nucleotide sequence for sec Tax mutant  polyA95
gctagcgtaatacgactcactataaggagacccaagctacatttgcttctgacacaactgtgttcactagcaacctcaaacagacaccgccaccatggactggacctggatcctgttcctggtggccgccgccacaagagtgcacagcgcacacttcccaggcttcggccagagcctgctgttcggctaccccgtgtacgtgttcggcgactgcgtgcaaggcgactggtgccccatcagcggcggcctgtgcagcgccagactgcacagacacgccctgctggccacatgccccgagcaccagatcacctgggaccccatcgacggcagagtgatcggaagcgccctgcagttcctgatccccagactgcccagcttccccacacagagaaccagcaagaccctgaaggtgctgaccccccccatcacacacaccacacccaacatccccccaagcttcctgcaggccatgcggaagtacagccccttcagaaacggctacatggaacccacactgggccagcacctgcccgccagcagcttccccgaccccggactgaggccccagaacctgtacacactgtggggcggcagcgtcgtgtgcatgtacctgtaccagctgagcccaccaatcacatggcccctgctgccccacgtgatcttctgccaccccggacagctgggcgccttcctgaccaacgtgccctacaagcggatcgaggaactgctgtacaagatcagcctgaccacaggcgccctgatcatcctgcccgaggactgcctgcccaccacactgttccagcccgccagagcccccgtgacactgaccgcctggcagaacggcctgctgccattccacagcaccctgacaacacccggcctgatctggaccttcaccgacggcacacccatgatcagcggcccctgccccaaggacggccagcccagcctggtgctgcagagcagcagcttcatcttccacaagttccagaccaaggcctaccaccccagcttcctgctgagccacggactgatccagtacagcagcttccacagcctgcacctgctgttcgaagagtacacaaacatccccatcagccggagcttcaacgagaaagaggccgacgacaacgaccacgagccccagatcagccccggcggactggaaccccccagcgagaagcacttccgggaaaccgaagtgtgagctcgctttcttgctgtccaatttctattaaaggttcctttgttccctaagtccaactactaaactgggggatattatgaagggccttgagcatctggattctgcctaataaaaaacatttattttcattgcaaaaaaaaaaaaaaaaaaaaaaaaaaaaaaaaaaaaaaaaaaaaaaaaaaaaaaaaaaaaaaaaaaaaaaaaaaaaaaaaaaaaaaaaaaaaaaacgaagagc

SEQ ID NO: 27 - DNA, 1427 bp, Artificial
  Template DNA nucleotide sequence for sec Tax mutant  polyA80
gctagcgtaatacgactcactataaggagacccaagctacatttgcttctgacacaactgtgttcactagcaacctcaaacagacaccgccaccatggactggacctggatcctgttcctggtggccgccgccacaagagtgcacagcgcacacttcccaggcttcggccagagcctgctgttcggctaccccgtgtacgtgttcggcgactgcgtgcaaggcgactggtgccccatcagcggcggcctgtgcagcgccagactgcacagacacgccctgctggccacatgccccgagcaccagatcacctgggaccccatcgacggcagagtgatcggaagcgccctgcagttcctgatccccagactgcccagcttccccacacagagaaccagcaagaccctgaaggtgctgaccccccccatcacacacaccacacccaacatccccccaagcttcctgcaggccatgcggaagtacagccccttcagaaacggctacatggaacccacactgggccagcacctgcccgccagcagcttccccgaccccggactgaggccccagaacctgtacacactgtggggcggcagcgtcgtgtgcatgtacctgtaccagctgagcccaccaatcacatggcccctgctgccccacgtgatcttctgccaccccggacagctgggcgccttcctgaccaacgtgccctacaagcggatcgaggaactgctgtacaagatcagcctgaccacaggcgccctgatcatcctgcccgaggactgcctgcccaccacactgttccagcccgccagagcccccgtgacactgaccgcctggcagaacggcctgctgccattccacagcaccctgacaacacccggcctgatctggaccttcaccgacggcacacccatgatcagcggcccctgccccaaggacggccagcccagcctggtgctgcagagcagcagcttcatcttccacaagttccagaccaaggcctaccaccccagcttcctgctgagccacggactgatccagtacagcagcttccacagcctgcacctgctgttcgaagagtacacaaacatccccatcagccggagcttcaacgagaaagaggccgacgacaacgaccacgagccccagatcagccccggcggactggaaccccccagcgagaagcacttccgggaaaccgaagtgtgagctcgctttcttgctgtccaatttctattaaaggttcctttgttccctaagtccaactactaaactgggggatattatgaagggccttgagcatctggattctgcctaataaaaaacatttattttcattgcaaaaaaaaaaaaaaaaaaaaaaaaaaaaaaaaaaaaaaaaaaaaaaaaaaaaaaaaaaaaaaaaaaaaaaaaaaaaaaaacgaagagc

SEQ ID NO: 28 - DNA, 1407 bp, Artificial
  Template DNA nucleotide sequence for sec Tax mutant  polyA60
gctagcgtaatacgactcactataaggagacccaagctacatttgcttctgacacaactgtgttcactagcaacctcaaacagacaccgccaccatggactggacctggatcctgttcctggtggccgccgccacaagagtgcacagcgcacacttcccaggcttcggccagagcctgctgttcggctaccccgtgtacgtgttcggcgactgcgtgcaaggcgactggtgccccatcagcggcggcctgtgcagcgccagactgcacagacacgccctgctggccacatgccccgagcaccagatcacctgggaccccatcgacggcagagtgatcggaagcgccctgcagttcctgatccccagactgcccagcttccccacacagagaaccagcaagaccctgaaggtgctgaccccccccatcacacacaccacacccaacatccccccaagcttcctgcaggccatgcggaagtacagccccttcagaaacggctacatggaacccacactgggccagcacctgcccgccagcagcttccccgaccccggactgaggccccagaacctgtacacactgtggggcggcagcgtcgtgtgcatgtacctgtaccagctgagcccaccaatcacatggcccctgctgccccacgtgatcttctgccaccccggacagctgggcgccttcctgaccaacgtgccctacaagcggatcgaggaactgctgtacaagatcagcctgaccacaggcgccctgatcatcctgcccgaggactgcctgcccaccacactgttccagcccgccagagcccccgtgacactgaccgcctggcagaacggcctgctgccattccacagcaccctgacaacacccggcctgatctggaccttcaccgacggcacacccatgatcagcggcccctgccccaaggacggccagcccagcctggtgctgcagagcagcagcttcatcttccacaagttccagaccaaggcctaccaccccagcttcctgctgagccacggactgatccagtacagcagcttccacagcctgcacctgctgttcgaagagtacacaaacatccccatcagccggagcttcaacgagaaagaggccgacgacaacgaccacgagccccagatcagccccggcggactggaaccccccagcgagaagcacttccgggaaaccgaagtgtgagctcgctttcttgctgtccaatttctattaaaggttcctttgttccctaagtccaactactaaactgggggatattatgaagggccttgagcatctggattctgcctaataaaaaacatttattttcattgcaaaaaaaaaaaaaaaaaaaaaaaaaaaaaaaaaaaaaaaaaaaaaaaaaaaaaaaaaaaacgaagagc

SEQ ID NO: 29 - DNA, 1387 bp, Artificial
  Template DNA nucleotide sequence for sec Tax mutant  polyA40
gctagcgtaatacgactcactataaggagacccaagctacatttgcttctgacacaactgtgttcactagcaacctcaaacagacaccgccaccatggactggacctggatcctgttcctggtggccgccgccacaagagtgcacagcgcacacttcccaggcttcggccagagcctgctgttcggctaccccgtgtacgtgttcggcgactgcgtgcaaggcgactggtgccccatcagcggcggcctgtgcagcgccagactgcacagacacgccctgctggccacatgccccgagcaccagatcacctgggaccccatcgacggcagagtgatcggaagcgccctgcagttcctgatccccagactgcccagcttccccacacagagaaccagcaagaccctgaaggtgctgaccccccccatcacacacaccacacccaacatccccccaagcttcctgcaggccatgcggaagtacagccccttcagaaacggctacatggaacccacactgggccagcacctgcccgccagcagcttccccgaccccggactgaggccccagaacctgtacacactgtggggcggcagcgtcgtgtgcatgtacctgtaccagctgagcccaccaatcacatggcccctgctgccccacgtgatcttctgccaccccggacagctgggcgccttcctgaccaacgtgccctacaagcggatcgaggaactgctgtacaagatcagcctgaccacaggcgccctgatcatcctgcccgaggactgcctgcccaccacactgttccagcccgccagagcccccgtgacactgaccgcctggcagaacggcctgctgccattccacagcaccctgacaacacccggcctgatctggaccttcaccgacggcacacccatgatcagcggcccctgccccaaggacggccagcccagcctggtgctgcagagcagcagcttcatcttccacaagttccagaccaaggcctaccaccccagcttcctgctgagccacggactgatccagtacagcagcttccacagcctgcacctgctgttcgaagagtacacaaacatccccatcagccggagcttcaacgagaaagaggccgacgacaacgaccacgagccccagatcagccccggcggactggaaccccccagcgagaagcacttccgggaaaccgaagtgtgagctcgctttcttgctgtccaatttctattaaaggttcctttgttccctaagtccaactactaaactgggggatattatgaagggccttgagcatctggattctgcctaataaaaaacatttattttcattgcaaaaaaaaaaaaaaaaaaaaaaaaaaaaaaaaaaaaaaaacgaagagc

SEQ ID NO: 30 - DNA, 1367 bp, Artificial
  Template DNA nucleotide sequence for sec Tax mutant  polyA20
gctagcgtaatacgactcactataaggagacccaagctacatttgcttctgacacaactgtgttcactagcaacctcaaacagacaccgccaccatggactggacctggatcctgttcctggtggccgccgccacaagagtgcacagcgcacacttcccaggcttcggccagagcctgctgttcggctaccccgtgtacgtgttcggcgactgcgtgcaaggcgactggtgccccatcagcggcggcctgtgcagcgccagactgcacagacacgccctgctggccacatgccccgagcaccagatcacctgggaccccatcgacggcagagtgatcggaagcgccctgcagttcctgatccccagactgcccagcttccccacacagagaaccagcaagaccctgaaggtgctgaccccccccatcacacacaccacacccaacatccccccaagcttcctgcaggccatgcggaagtacagccccttcagaaacggctacatggaacccacactgggccagcacctgcccgccagcagcttccccgaccccggactgaggccccagaacctgtacacactgtggggcggcagcgtcgtgtgcatgtacctgtaccagctgagcccaccaatcacatggcccctgctgccccacgtgatcttctgccaccccggacagctgggcgccttcctgaccaacgtgccctacaagcggatcgaggaactgctgtacaagatcagcctgaccacaggcgccctgatcatcctgcccgaggactgcctgcccaccacactgttccagcccgccagagcccccgtgacactgaccgcctggcagaacggcctgctgccattccacagcaccctgacaacacccggcctgatctggaccttcaccgacggcacacccatgatcagcggcccctgccccaaggacggccagcccagcctggtgctgcagagcagcagcttcatcttccacaagttccagaccaaggcctaccaccccagcttcctgctgagccacggactgatccagtacagcagcttccacagcctgcacctgctgttcgaagagtacacaaacatccccatcagccggagcttcaacgagaaagaggccgacgacaacgaccacgagccccagatcagccccggcggactggaaccccccagcgagaagcacttccgggaaaccgaagtgtgagctcgctttcttgctgtccaatttctattaaaggttcctttgttccctaagtccaactactaaactgggggatattatgaagggccttgagcatctggattctgcctaataaaaaacatttattttcattgcaaaaaaaaaaaaaaaaaaaacgaagagc

SEQ ID NO: 31 - RNA, 1317 nt, Artificial
  mRNA sequence for gp46-Fib  polyA95
aggagacccaagcuacauuugcuucugacacaacuguguucacuagcaaccucaaacagacaccgccaccaugggcaaguuccuggccacacugauccuguucuuccaguucugcccccugaucuucggcgacuacagccccagcugcugcacccugacaaucggcgugagcagcuaccacagcaagcccugcaaccccgcccagcccgugugcagcuggacccuggaccugcuggcccugagcgccgaccaggcccugcagccccccugccccaaccuggugagcuacagcagcuaccacgccaccuacagccuguaccuguucccccacuggaccaagaagcccaacagaaacggcggaggcuacuacagcgccagcuacagcgaccccugcagccugaagugccccuaccugggcugccagagcuggacaugccccuacacaggcgccgugagcagccccuacuggaaguuccagcacgacgugaacuucacccaagaggugagccggcugaacaucaaccugcacuucagcaagugcggcuucccauucagccugcugguggacgcccccggcuacgaccccaucugguuccugaacaccgagcccagccagcugcccccaacagccccaccccugcugccccacagcaaccuggaccacauccuggaacccagcauccccuggaagagcaagcugcugacacuggugcagcugacccugcagagcaccaacuacaccugcaucgugugcaucgaccgggccagccugagcacauggcacgugcuguacagccccaacgugagcgugcccagcagcagcagcacaccccugcuguaccccagccuggcacugcccgccccccaccugacacugcccuucaacuggacccacugcuucgacccccagauccaggccaucgugagcagcccaugccacaacagccugauccugcccccauucagccugagccccgugcccacacucggcagcggcagcggcagcggcuacauccccgaggcccccagagacggccaggccuacgucagaaaggacggcgaaugggugcugcugagcaccuuccugugagcucgcuuucuugcuguccaauuucuauuaaagguuccuuuguucccuaaguccaacuacuaaacugggggauauuaugaagggccuugagcaucuggauucugccuaauaaaaaacauuuauuuucauugcaaaaaaaaaaaaaaaaaaaaaaaaaaaaaaaaaaaaaaaaaaaaaaaaaaaaaaaaaaaaaaaaaaaaaaaaaaaaaaaaaaaaaaaaaaaaaaa

SEQ ID NO: 32 - RNA, 1302 nt, Artificial
  mRNA sequence for gp46-Fib  polyA80
aggagacccaagcuacauuugcuucugacacaacuguguucacuagcaaccucaaacagacaccgccaccaugggcaaguuccuggccacacugauccuguucuuccaguucugcccccugaucuucggcgacuacagccccagcugcugcacccugacaaucggcgugagcagcuaccacagcaagcccugcaaccccgcccagcccgugugcagcuggacccuggaccugcuggcccugagcgccgaccaggcccugcagccccccugccccaaccuggugagcuacagcagcuaccacgccaccuacagccuguaccuguucccccacuggaccaagaagcccaacagaaacggcggaggcuacuacagcgccagcuacagcgaccccugcagccugaagugccccuaccugggcugccagagcuggacaugccccuacacaggcgccgugagcagccccuacuggaaguuccagcacgacgugaacuucacccaagaggugagccggcugaacaucaaccugcacuucagcaagugcggcuucccauucagccugcugguggacgcccccggcuacgaccccaucugguuccugaacaccgagcccagccagcugcccccaacagccccaccccugcugccccacagcaaccuggaccacauccuggaacccagcauccccuggaagagcaagcugcugacacuggugcagcugacccugcagagcaccaacuacaccugcaucgugugcaucgaccgggccagccugagcacauggcacgugcuguacagccccaacgugagcgugcccagcagcagcagcacaccccugcuguaccccagccuggcacugcccgccccccaccugacacugcccuucaacuggacccacugcuucgacccccagauccaggccaucgugagcagcccaugccacaacagccugauccugcccccauucagccugagccccgugcccacacucggcagcggcagcggcagcggcuacauccccgaggcccccagagacggccaggccuacgucagaaaggacggcgaaugggugcugcugagcaccuuccugugagcucgcuuucuugcuguccaauuucuauuaaagguuccuuuguucccuaaguccaacuacuaaacugggggauauuaugaagggccuugagcaucuggauucugccuaauaaaaaacauuuauuuucauugcaaaaaaaaaaaaaaaaaaaaaaaaaaaaaaaaaaaaaaaaaaaaaaaaaaaaaaaaaaaaaaaaaaaaaaaaaaaaaaaa

SEQ ID NO: 33 - RNA, 1282 nt, Artificial
  mRNA sequence for gp46-Fib  polyA60
aggagacccaagcuacauuugcuucugacacaacuguguucacuagcaaccucaaacagacaccgccaccaugggcaaguuccuggccacacugauccuguucuuccaguucugcccccugaucuucggcgacuacagccccagcugcugcacccugacaaucggcgugagcagcuaccacagcaagcccugcaaccccgcccagcccgugugcagcuggacccuggaccugcuggcccugagcgccgaccaggcccugcagccccccugccccaaccuggugagcuacagcagcuaccacgccaccuacagccuguaccuguucccccacuggaccaagaagcccaacagaaacggcggaggcuacuacagcgccagcuacagcgaccccugcagccugaagugccccuaccugggcugccagagcuggacaugccccuacacaggcgccgugagcagccccuacuggaaguuccagcacgacgugaacuucacccaagaggugagccggcugaacaucaaccugcacuucagcaagugcggcuucccauucagccugcugguggacgcccccggcuacgaccccaucugguuccugaacaccgagcccagccagcugcccccaacagccccaccccugcugccccacagcaaccuggaccacauccuggaacccagcauccccuggaagagcaagcugcugacacuggugcagcugacccugcagagcaccaacuacaccugcaucgugugcaucgaccgggccagccugagcacauggcacgugcuguacagccccaacgugagcgugcccagcagcagcagcacaccccugcuguaccccagccuggcacugcccgccccccaccugacacugcccuucaacuggacccacugcuucgacccccagauccaggccaucgugagcagcccaugccacaacagccugauccugcccccauucagccugagccccgugcccacacucggcagcggcagcggcagcggcuacauccccgaggcccccagagacggccaggccuacgucagaaaggacggcgaaugggugcugcugagcaccuuccugugagcucgcuuucuugcuguccaauuucuauuaaagguuccuuuguucccuaaguccaacuacuaaacugggggauauuaugaagggccuugagcaucuggauucugccuaauaaaaaacauuuauuuucauugcaaaaaaaaaaaaaaaaaaaaaaaaaaaaaaaaaaaaaaaaaaaaaaaaaaaaaaaaaaaa

SEQ ID NO: 34 - RNA, 1262 nt, Artificial
  mRNA sequence for gp46-Fib  polyA95
aggagacccaagcuacauuugcuucugacacaacuguguucacuagcaaccucaaacagacaccgccaccaugggcaaguuccuggccacacugauccuguucuuccaguucugcccccugaucuucggcgacuacagccccagcugcugcacccugacaaucggcgugagcagcuaccacagcaagcccugcaaccccgcccagcccgugugcagcuggacccuggaccugcuggcccugagcgccgaccaggcccugcagccccccugccccaaccuggugagcuacagcagcuaccacgccaccuacagccuguaccuguucccccacuggaccaagaagcccaacagaaacggcggaggcuacuacagcgccagcuacagcgaccccugcagccugaagugccccuaccugggcugccagagcuggacaugccccuacacaggcgccgugagcagccccuacuggaaguuccagcacgacgugaacuucacccaagaggugagccggcugaacaucaaccugcacuucagcaagugcggcuucccauucagccugcugguggacgcccccggcuacgaccccaucugguuccugaacaccgagcccagccagcugcccccaacagccccaccccugcugccccacagcaaccuggaccacauccuggaacccagcauccccuggaagagcaagcugcugacacuggugcagcugacccugcagagcaccaacuacaccugcaucgugugcaucgaccgggccagccugagcacauggcacgugcuguacagccccaacgugagcgugcccagcagcagcagcacaccccugcuguaccccagccuggcacugcccgccccccaccugacacugcccuucaacuggacccacugcuucgacccccagauccaggccaucgugagcagcccaugccacaacagccugauccugcccccauucagccugagccccgugcccacacucggcagcggcagcggcagcggcuacauccccgaggcccccagagacggccaggccuacgucagaaaggacggcgaaugggugcugcugagcaccuuccugugagcucgcuuucuugcuguccaauuucuauuaaagguuccuuuguucccuaaguccaacuacuaaacugggggauauuaugaagggccuugagcaucuggauucugccuaauaaaaaacauuuauuuucauugcaaaaaaaaaaaaaaaaaaaaaaaaaaaaaaaaaaaaaaaa

SEQ ID NO: 35 - RNA, 1242 nt, Artificial
  mRNA sequence for gp46-Fib  polyA20
aggagacccaagcuacauuugcuucugacacaacuguguucacuagcaaccucaaacagacaccgccaccaugggcaaguuccuggccacacugauccuguucuuccaguucugcccccugaucuucggcgacuacagccccagcugcugcacccugacaaucggcgugagcagcuaccacagcaagcccugcaaccccgcccagcccgugugcagcuggacccuggaccugcuggcccugagcgccgaccaggcccugcagccccccugccccaaccuggugagcuacagcagcuaccacgccaccuacagccuguaccuguucccccacuggaccaagaagcccaacagaaacggcggaggcuacuacagcgccagcuacagcgaccccugcagccugaagugccccuaccugggcugccagagcuggacaugccccuacacaggcgccgugagcagccccuacuggaaguuccagcacgacgugaacuucacccaagaggugagccggcugaacaucaaccugcacuucagcaagugcggcuucccauucagccugcugguggacgcccccggcuacgaccccaucugguuccugaacaccgagcccagccagcugcccccaacagccccaccccugcugccccacagcaaccuggaccacauccuggaacccagcauccccuggaagagcaagcugcugacacuggugcagcugacccugcagagcaccaacuacaccugcaucgugugcaucgaccgggccagccugagcacauggcacgugcuguacagccccaacgugagcgugcccagcagcagcagcacaccccugcuguaccccagccuggcacugcccgccccccaccugacacugcccuucaacuggacccacugcuucgacccccagauccaggccaucgugagcagcccaugccacaacagccugauccugcccccauucagccugagccccgugcccacacucggcagcggcagcggcagcggcuacauccccgaggcccccagagacggccaggccuacgucagaaaggacggcgaaugggugcugcugagcaccuuccugugagcucgcuuucuugcuguccaauuucuauuaaagguuccuuuguucccuaaguccaacuacuaaacugggggauauuaugaagggccuugagcaucuggauucugccuaauaaaaaacauuuauuuucauugcaaaaaaaaaaaaaaaaaaaa

SEQ ID NO: 36 - RNA, 1410 nt, Artificial
  mRNA sequence for sec Tax mutant  polyA95
aggagacccaagcuacauuugcuucugacacaacuguguucacuagcaaccucaaacagacaccgccaccauggacuggaccuggauccuguuccugguggccgccgccacaagagugcacagcgcacacuucccaggcuucggccagagccugcuguucggcuaccccguguacguguucggcgacugcgugcaaggcgacuggugccccaucagcggcggccugugcagcgccagacugcacagacacgcccugcuggccacaugccccgagcaccagaucaccugggaccccaucgacggcagagugaucggaagcgcccugcaguuccugauccccagacugcccagcuuccccacacagagaaccagcaagacccugaaggugcugaccccccccaucacacacaccacacccaacauccccccaagcuuccugcaggccaugcggaaguacagccccuucagaaacggcuacauggaacccacacugggccagcaccugcccgccagcagcuuccccgaccccggacugaggccccagaaccuguacacacuguggggcggcagcgucgugugcauguaccuguaccagcugagcccaccaaucacauggccccugcugccccacgugaucuucugccaccccggacagcugggcgccuuccugaccaacgugcccuacaagcggaucgaggaacugcuguacaagaucagccugaccacaggcgcccugaucauccugcccgaggacugccugcccaccacacuguuccagcccgccagagcccccgugacacugaccgccuggcagaacggccugcugccauuccacagcacccugacaacacccggccugaucuggaccuucaccgacggcacacccaugaucagcggccccugccccaaggacggccagcccagccuggugcugcagagcagcagcuucaucuuccacaaguuccagaccaaggccuaccaccccagcuuccugcugagccacggacugauccaguacagcagcuuccacagccugcaccugcuguucgaagaguacacaaacauccccaucagccggagcuucaacgagaaagaggccgacgacaacgaccacgagccccagaucagccccggcggacuggaaccccccagcgagaagcacuuccgggaaaccgaagugugagcucgcuuucuugcuguccaauuucuauuaaagguuccuuuguucccuaaguccaacuacuaaacugggggauauuaugaagggccuugagcaucuggauucugccuaauaaaaaacauuuauuuucauugcaaaaaaaaaaaaaaaaaaaaaaaaaaaaaaaaaaaaaaaaaaaaaaaaaaaaaaaaaaaaaaaaaaaaaaaaaaaaaaaaaaaaaaaaaaaaaaa

SEQ ID NO: 37 - RNA, 1395 nt, Artificial
  mRNA sequence for sec Tax mutant  polyA80
aggagacccaagcuacauuugcuucugacacaacuguguucacuagcaaccucaaacagacaccgccaccauggacuggaccuggauccuguuccugguggccgccgccacaagagugcacagcgcacacuucccaggcuucggccagagccugcuguucggcuaccccguguacguguucggcgacugcgugcaaggcgacuggugccccaucagcggcggccugugcagcgccagacugcacagacacgcccugcuggccacaugccccgagcaccagaucaccugggaccccaucgacggcagagugaucggaagcgcccugcaguuccugauccccagacugcccagcuuccccacacagagaaccagcaagacccugaaggugcugaccccccccaucacacacaccacacccaacauccccccaagcuuccugcaggccaugcggaaguacagccccuucagaaacggcuacauggaacccacacugggccagcaccugcccgccagcagcuuccccgaccccggacugaggccccagaaccuguacacacuguggggcggcagcgucgugugcauguaccuguaccagcugagcccaccaaucacauggccccugcugccccacgugaucuucugccaccccggacagcugggcgccuuccugaccaacgugcccuacaagcggaucgaggaacugcuguacaagaucagccugaccacaggcgcccugaucauccugcccgaggacugccugcccaccacacuguuccagcccgccagagcccccgugacacugaccgccuggcagaacggccugcugccauuccacagcacccugacaacacccggccugaucuggaccuucaccgacggcacacccaugaucagcggccccugccccaaggacggccagcccagccuggugcugcagagcagcagcuucaucuuccacaaguuccagaccaaggccuaccaccccagcuuccugcugagccacggacugauccaguacagcagcuuccacagccugcaccugcuguucgaagaguacacaaacauccccaucagccggagcuucaacgagaaagaggccgacgacaacgaccacgagccccagaucagccccggcggacuggaaccccccagcgagaagcacuuccgggaaaccgaagugugagcucgcuuucuugcuguccaauuucuauuaaagguuccuuuguucccuaaguccaacuacuaaacugggggauauuaugaagggccuugagcaucuggauucugccuaauaaaaaacauuuauuuucauugcaaaaaaaaaaaaaaaaaaaaaaaaaaaaaaaaaaaaaaaaaaaaaaaaaaaaaaaaaaaaaaaaaaaaaaaaaaaaaaaa

SEQ ID NO: 38 - RNA, 1375 nt, Artificial
  mRNA sequence for sec Tax mutant  polyA60
aggagacccaagcuacauuugcuucugacacaacuguguucacuagcaaccucaaacagacaccgccaccauggacuggaccuggauccuguuccugguggccgccgccacaagagugcacagcgcacacuucccaggcuucggccagagccugcuguucggcuaccccguguacguguucggcgacugcgugcaaggcgacuggugccccaucagcggcggccugugcagcgccagacugcacagacacgcccugcuggccacaugccccgagcaccagaucaccugggaccccaucgacggcagagugaucggaagcgcccugcaguuccugauccccagacugcccagcuuccccacacagagaaccagcaagacccugaaggugcugaccccccccaucacacacaccacacccaacauccccccaagcuuccugcaggccaugcggaaguacagccccuucagaaacggcuacauggaacccacacugggccagcaccugcccgccagcagcuuccccgaccccggacugaggccccagaaccuguacacacuguggggcggcagcgucgugugcauguaccuguaccagcugagcccaccaaucacauggccccugcugccccacgugaucuucugccaccccggacagcugggcgccuuccugaccaacgugcccuacaagcggaucgaggaacugcuguacaagaucagccugaccacaggcgcccugaucauccugcccgaggacugccugcccaccacacuguuccagcccgccagagcccccgugacacugaccgccuggcagaacggccugcugccauuccacagcacccugacaacacccggccugaucuggaccuucaccgacggcacacccaugaucagcggccccugccccaaggacggccagcccagccuggugcugcagagcagcagcuucaucuuccacaaguuccagaccaaggccuaccaccccagcuuccugcugagccacggacugauccaguacagcagcuuccacagccugcaccugcuguucgaagaguacacaaacauccccaucagccggagcuucaacgagaaagaggccgacgacaacgaccacgagccccagaucagccccggcggacuggaaccccccagcgagaagcacuuccgggaaaccgaagugugagcucgcuuucuugcuguccaauuucuauuaaagguuccuuuguucccuaaguccaacuacuaaacugggggauauuaugaagggccuugagcaucuggauucugccuaauaaaaaacauuuauuuucauugcaaaaaaaaaaaaaaaaaaaaaaaaaaaaaaaaaaaaaaaaaaaaaaaaaaaaaaaaaaaa

SEQ ID NO: 39 - RNA, 1355 nt, Artificial
  mRNA sequence for sec Tax mutant  polyA40
aggagacccaagcuacauuugcuucugacacaacuguguucacuagcaaccucaaacagacaccgccaccauggacuggaccuggauccuguuccugguggccgccgccacaagagugcacagcgcacacuucccaggcuucggccagagccugcuguucggcuaccccguguacguguucggcgacugcgugcaaggcgacuggugccccaucagcggcggccugugcagcgccagacugcacagacacgcccugcuggccacaugccccgagcaccagaucaccugggaccccaucgacggcagagugaucggaagcgcccugcaguuccugauccccagacugcccagcuuccccacacagagaaccagcaagacccugaaggugcugaccccccccaucacacacaccacacccaacauccccccaagcuuccugcaggccaugcggaaguacagccccuucagaaacggcuacauggaacccacacugggccagcaccugcccgccagcagcuuccccgaccccggacugaggccccagaaccuguacacacuguggggcggcagcgucgugugcauguaccuguaccagcugagcccaccaaucacauggccccugcugccccacgugaucuucugccaccccggacagcugggcgccuuccugaccaacgugcccuacaagcggaucgaggaacugcuguacaagaucagccugaccacaggcgcccugaucauccugcccgaggacugccugcccaccacacuguuccagcccgccagagcccccgugacacugaccgccuggcagaacggccugcugccauuccacagcacccugacaacacccggccugaucuggaccuucaccgacggcacacccaugaucagcggccccugccccaaggacggccagcccagccuggugcugcagagcagcagcuucaucuuccacaaguuccagaccaaggccuaccaccccagcuuccugcugagccacggacugauccaguacagcagcuuccacagccugcaccugcuguucgaagaguacacaaacauccccaucagccggagcuucaacgagaaagaggccgacgacaacgaccacgagccccagaucagccccggcggacuggaaccccccagcgagaagcacuuccgggaaaccgaagugugagcucgcuuucuugcuguccaauuucuauuaaagguuccuuuguucccuaaguccaacuacuaaacugggggauauuaugaagggccuugagcaucuggauucugccuaauaaaaaacauuuauuuucauugcaaaaaaaaaaaaaaaaaaaaaaaaaaaaaaaaaaaaaaaa

SEQ ID NO: 40 - RNA, 1335 nt, Artificial
  mRNA sequence for sec Tax mutant  polyA20
aggagacccaagcuacauuugcuucugacacaacuguguucacuagcaaccucaaacagacaccgccaccauggacuggaccuggauccuguuccugguggccgccgccacaagagugcacagcgcacacuucccaggcuucggccagagccugcuguucggcuaccccguguacguguucggcgacugcgugcaaggcgacuggugccccaucagcggcggccugugcagcgccagacugcacagacacgcccugcuggccacaugccccgagcaccagaucaccugggaccccaucgacggcagagugaucggaagcgcccugcaguuccugauccccagacugcccagcuuccccacacagagaaccagcaagacccugaaggugcugaccccccccaucacacacaccacacccaacauccccccaagcuuccugcaggccaugcggaaguacagccccuucagaaacggcuacauggaacccacacugggccagcaccugcccgccagcagcuuccccgaccccggacugaggccccagaaccuguacacacuguggggcggcagcgucgugugcauguaccuguaccagcugagcccaccaaucacauggccccugcugccccacgugaucuucugccaccccggacagcugggcgccuuccugaccaacgugcccuacaagcggaucgaggaacugcuguacaagaucagccugaccacaggcgcccugaucauccugcccgaggacugccugcccaccacacuguuccagcccgccagagcccccgugacacugaccgccuggcagaacggccugcugccauuccacagcacccugacaacacccggccugaucuggaccuucaccgacggcacacccaugaucagcggccccugccccaaggacggccagcccagccuggugcugcagagcagcagcuucaucuuccacaaguuccagaccaaggccuaccaccccagcuuccugcugagccacggacugauccaguacagcagcuuccacagccugcaccugcuguucgaagaguacacaaacauccccaucagccggagcuucaacgagaaagaggccgacgacaacgaccacgagccccagaucagccccggcggacuggaaccccccagcgagaagcacuuccgggaaaccgaagugugagcucgcuuucuugcuguccaauuucuauuaaagguuccuuuguucccuaaguccaacuacuaaacugggggauauuaugaagggccuugagcaucuggauucugccuaauaaaaaacauuuauuuucauugcaaaaaaaaaaaaaaaaaaaa